European Patent Specification EP 3 364 985 B1, published February 11, 2026. Title: Methods for Generating Engineered Human Primary Blood Dendritic Cell Lines. Applicant: University of Maryland, Baltimore. The sequence listing filed with the application follows.

SEQUENCE LISTING (54 sequences)

SEQ ID NO: 1 - protein, 353 aa, HTLV-1
MAHFPGFGQSLLFGYPVYVFGDCVQGDWCPISGGLCSARLHRHALLATCPEHQITWDPIDGRVIGSALQFLIPRLPSFPTQRTSKTLKVLTPPITHTTPNIPPSFLQAMRKYSPFRNGYMEPTLGQHLPTLSFPDPGLRPQNLYTLWGGSVVCMYLYQLSPPITWPLLPHVIFCHPGQLGAFLTNVPYKRIEELLYKISLTTGALIILPEDCLPTTLFQPARAPVTLTAWQNGLLPFHSTLTTPGLIWTFTDGTPMISGPCPKDGQPSLVLQSSSFIFHKFQTKAYHPSFLLSHGLIQYSSFHSLHLLFEEYTNIPISLLFNEKEADDNDHEPQISPGGLEPPSEKHFRETEV

SEQ ID NO: 2 - DNA, 1062 bp, HTLV-1
atggcccatttcccagggtttggacagagtcttcttttcggatacccagtctacgtgtttggagactgtgtacaaggcgactggtgccccatctctgggggactatgttcggcccgcctacatcgtcacgccctactggccacctgtccagagcatcagatcacctgggaccccatcgacggacgcgttatcggctcagctctacagttccttatccctcgactcccctccttccccacccagagaacctctaagaccctcaaggtccttaccccgccaatcactcatacaacccccaacattccaccctccttcctccaggccatgcgcaaatactcccccttccgaaatggatacatggaacccacccttgggcagcacctcccaaccctgtcttttccagaccccggactccggccccaaaacctgtacaccctctggggaggctccgttgtctgcatgtacctctaccagctttccccccccatcacctggcccctcctgccccacgtgattttttgccaccccggccagctcggggccttcctcaccaatgttccctacaagcgaatagaagaactcctctataaaatttccctcaccacaggggccctaataattctacccgaagactgtttgcccaccacccttttccagcctgctagggcacccgtcacgctaacagcctggcaaaacggcctccttccgttccactcaaccctcaccactccaggccttatttggacatttaccgatggcacgcctatgatttccgggccctgccctaaagatggccagccatctttagtactacagtcctcctcctttatatttcacaaatttcaaaccaaggcctaccacccctcatttctactctcacacggcctcatacagtactcttcctttcatagtttacatctcctgtttgaagaatacaccaacatccccatttctctactttttaacgaaaaagaggcagatgacaatgaccatgagccccaaatatcccccgggggcttagagcctcccagtgaaaaacatttccgagaaacagaagtctga

SEQ ID NO: 3 - protein, 331 aa, HTLV-2
MAHFPGFGQSLLYGYPVYVFGDCVQADWCPVSGGLCSTRLHRHALLATCPEHQLTWDPIDGRVVSSPLQYLIPRLPSFPTQRTSRTLKVLTPPTTPVSPKVPPAFFQSMRKHTPYRNGCLEPTLGDQLPSLAFPEPGLRPQNIYTTWGKTVVCLYLYQLSPPMTWPLIPHVIFCHPRQLGAFLTKVPLKRLEELLYKMFLHTGTVIVLPVDDLPTTMFQPVRAPCIQTAWCTGLLPYHSILTTPGLIWTFNDGSPMISGPCPKAGQPSLVVQSSLLIFEKFQTKAFHPSYLLSHQLIQYSSFHNLHLLFDEYTNIPVSILFNKEEADDNGD

SEQ ID NO: 4 - DNA, 996 bp, HTLV-2
atggcccatttcccaggatttggacaaagcctcctatatggataccccgtctacgtgtttggcgattgtgtacaggccgattggtgtcccgtctcaggtggtctatgttccacccgcctacatcgacatgccctcctggccacctgtccagagcaccaactcacctgggaccccatcgatggacgcgttgtcagctctcctctccaataccttatccctcgcctcccctccttccccacccagagaacctcaaggaccctcaaggtccttacccctcccaccactcctgtctcccccaaggttccacctgccttctttcaatcaatgcgaaagcacaccccctaccgaaatggatgcctggaaccaaccctcggggatcagctcccctccctcgccttccccgaacctggcctccgtccccaaaacatctacaccacctggggaaaaaccgtagtatgcctatacctataccagctttccccacccatgacatggccacttataccccatgtcatattctgccaccccagacaattaggagccttcctcaccaaggtgcctctaaaacgattagaagaacttctatacaaaatgttcctacacacagggacagtcatagtcctcccagtggacgacctacccaccacaatgttccaacccgtgagggctccctgtatccagactgcctggtgtacaggacttctcccctatcactccatcttaacaaccccaggtctaatatggaccttcaatgacggctcaccaatgatttccggcccttgccccaaagcagggcagccatctttagtagttcagtcctccctattaatcttcgaaaaattccaaaccaaagccttccatccctcctatctactctctcatcagcttatacaatactcctccttccataaccttcaccttctattcgatgaatacaccaacatccctgtctctattttatttaataaagaagaggcggatgacaatggcgactga

SEQ ID NO: 5 - protein, 350 aa, HTLV-3
MAHFPGFGQSLLYGYPVYVFGDCVQADWCPISGGLCSARLHRHALLATCPEHQITWDPIDGRVVSSALQYLIPRLPSFPTQRTTRTLKVLTPPTTAATPKIPPSFFHAVKKHTPFRNNCLELTLGEQLPAMSFPDPGLRPQNIYTMWGSSVVCLYLYQLSPPMTWPLIPHVIFCHPEQLGAFLTRVPTKRLEELLYKIFLSTGAIIILPENCFPTTLFQPTRAPAVQAPWHTGLLPCQKEIATPGLIWTFTDGSPMISGPCPKEGQPSLVVQSSTFIFQQFQTKASHPAFLLSHKLIHYSSFHSLHLLFEEYTTIPFSLLFNEKGANVDDDEPRDGSQPPARGQIAESPV

SEQ ID NO: 6 - DNA, 1053 bp, HTLV-3
atggcccatttcccaggtttcggacagagccttctctacgggtaccctgtctacgttttcggcgactgtgtacaggccgattggtgccccatttctggggggctttgttccgctcggctacaccgccatgccctactggccacgtgccccgaacatcagattacctgggaccccatcgatggacgcgttgtcagctcagctctacaataccttatccctcgactcccctccttccccacccagagaactacccgcaccctcaaggttctcacccccccaaccactgctgcgacccccaagattcctccatccttcttccacgccgttaaaaaacacacccccttccgaaacaattgccttgaactcaccctgggagagcagttgccagccatgtccttccccgaccctgggctccgaccccaaaacatctacaccatgtggggaagctccgttgtgtgcctttacctctatcagctctccccccccatgacctggcctctaatcccgcatgttatattctgccatcctgagcagcttggagccttcctcacccgagtccctaccaaacgattagaagaactcctgtataagatatttttaagcacaggggcgataatcatcctgcctgaaaactgttttccaaccaccctgttccaacccacccgcgcgcccgcggtgcaggccccctggcacacaggcctgctcccgtgtcaaaaggaaattgctacccccgggctcatttggactttcactgatggcagccccatgatttccggcccttgccccaaagaaggacagccatctttagtagtacaatcatctacatttatctttcaacaattccaaaccaaggccagtcaccccgctttcctcttgtcccacaaactaatccactactcctcttttcattccctccacctcctctttgaggaatatacaactatccccttttctctactttttaatgaaaaaggggcaaatgtcgatgatgatgagccccgagacgggtcacaaccaccagctagaggacaaatagctgagtcacccgtctga

SEQ ID NO: 7 - protein, 345 aa, HTLV-4
MAHFPGFGQSLLYGYPVYVFGDCVQADWCPISGGLCSPRLHRHALLATCPEHQITWDPIDGRVVGSPLQYLIPRLPSFPTQRTSKTLKVLTPPTTPVTPKVPPSFFQSVRRHSPYRNGCLETTLGEQLPSLAFPEPGLRPQNVYTIWGKTIVCLYIYQLSPPMTWPLIPHVIFCNPRQLGAFLSNVPPKRLEELLYKLYLHTGAIIILPEDALPTTLFQPVRAPCVQTTWNTGLLPYQPNLTTPGLIWTFNDGSPMISGPCPKAGQPSLVVQSSLLIFERFQTKAYHPSYLLSHQLIQYSSFHHLYLLFDEYTTIPFSLLFKEKEGDDRDNDPLPGATASPQGQN

SEQ ID NO: 8 - DNA, 1038 bp, HTLV-4
atggcccacttcccaggattcgggcagagcctcctctatggataccccgtctatgtgtttggcgattgtgttcaagccgattggtgccccatctccggtggattatgctccccccgcctacatcgccacgccctcctggccacctgccccgagcaccagatcacctgggaccccatcgatggacgagttgtcggctcgcctctccaataccttatccctcgcctcccctccttccccacccaacgaacctccaagaccctcaaagtccttaccccaccaaccactcctgtcacccccaaggttccaccctccttctttcagtccgtgcggaggcacagcccctaccgcaacggatgtcttgaaacaacccttggagagcagctcccctcccttgcatttcctgagccaggcctcaggccccaaaacgtctacaccatctggggaaagaccatagtgtgtctatacatctaccagctgtcccctcccatgacctggcccctcattccccatgtcatattttgcaaccccaggcagcttggcgcttttctaagcaatgtgccccccaagcgattagaagaactcctctacaaactttatctacacaccggcgccataatcatcctgccggaagacgccctgcctaccaccctatttcagcctgttcgagcaccctgtgtccaaactacctggaacacaggacttctcccataccagccaaacctgactacccctggcctgatatggacctttaatgatgggtctcctatgatttcaggaccttgccctaaggcagggcagccatccttggtagtacagtcctcactactaatcttcgagagatttcaaaccaaagcctatcatccctcttacctcctctcccaccaattgatacagtattcctccttccatcacctctacttactctttgatgaatatactactatccccttctctctactatttaaggaaaaagagggagatgacagggacaacgaccctctcccaggggcgacagcaagcccccaaggacaaaactag

SEQ ID NO: 9 - protein, 1069 aa, Homo sapiens
MPRAPRCRAVRSLLRSHYREVLPLATFVRRLGPQGWRLVQRGDPAAFRALVAQCLVCVPWDARPPPAAPSFRQVSCLKELVARVLQRLCERGAKNVLAFGFALLDGARGGPPEAFTTSVRSYLPNTVTDALRGSGAWGLLLRRVGDDVLVHLLARCALFVLVAPSCAYQVCGPPLYQLGAATQARPPPHASGPRRRLGCERAWNHSVREAGVPLGLPAPGARRRGGSASRSLPLPKRPRRGAAPEPERTPVGQGSWAHPGRTRGPSDRGFCVVSPARPAEEATSLEGALSGTRHSHPSVGRQHHAGPPSTSRPPRPWDTPCPPVYAETKHFLYSSGDKEQLRPSFLLSSLRPSLTGARRLVETIFLGSRPWMPGTPRRLPRLPQRYWQMRPLFLELLGNHAQCPYGVLLKTHCPLRAAVTPAAGVCAREKPQGSVAAPEEEDTDPRRLVQLLRQHSSPWQVYGFVRACLRRLVPPGLWGSRHNERRFLRNTKKFISLGKHAKLSLQELTWKMSVRDCAWLRRSPGVGCVPAAEHRLREEILAKFLHWLMSVYVVELLRSFFYVTETTFQKNRLFFYRKSVWSKLQSIGIRQHLKRVQLRELSEAEVRQHREARPALLTSRLRFIPKPDGLRPIVNMDYVVGARTFRREKRAERLTSRVKALFSVLNYERARRPGLLGASVLGLDDIHRAWRTFVLRVRAQDPPPELYFVKVDVTGAYDTIPQDRLTEVIASIIKPQNTYCVRRYAVVQKAAHGHVRKAFKSHVSTLTDLQPYMRQFVAHLQETSPLRDAVVIEQSSSLNEASSGLFDVFLRFMCHHAVRIRGKSYVQCQGIPQGSILSTLLCSLCYGDMENKLFAGIRRDGLLLRLVDDFLLVTPHLTHAKTFLSYARTSIRASLTFNRGFKAGRNMRRKLFGVLRLKCHSLFLDLQVNSLQTVCTNIYKILLLQAYRFHACVLQLPFHQQVWKNPTFFLRVISDTASLCYSILKAKNAGMSLGAKGAAGPLPSEAVQWLCHQAFLLKLTRHRVTYVPLLGSLRTAQTQLSRKLPGTTLTALEAAANPALPSDFKTILD

SEQ ID NO: 10 - DNA, 3210 bp, Homo sapiens
atgccgcgcgctccccgctgccgagccgtgcgctccctgctgcgcagccactaccgcgaggtgctgccgctggccacgttcgtgcggcgcctggggccccagggctggcggctggtgcagcgcggggacccggcggctttccgcgcgctggtggcccagtgcctggtgtgcgtgccctgggacgcacggccgccccccgccgccccctccttccgccaggtgtcctgcctgaaggagctggtggcccgagtgctgcagaggctgtgcgagcgcggcgcgaagaacgtgctggccttcggcttcgcgctgctggacggggcccgcgggggcccccccgaggccttcaccaccagcgtgcgcagctacctgcccaacacggtgaccgacgcactgcgggggagcggggcgtgggggctgctgctgcgccgcgtgggcgacgacgtgctggttcacctgctggcacgctgcgcgctctttgtgctggtggctcccagctgcgcctaccaggtgtgcgggccgccgctgtaccagctcggcgctgccactcaggcccggcccccgccacacgctagtggaccccgaaggcgtctgggatgcgaacgggcctggaaccatagcgtcagggaggccggggtccccctgggcctgccagccccgggtgcgaggaggcgcgggggcagtgccagccgaagtctgccgttgcccaagaggcccaggcgtggcgctgcccctgagccggagcggacgcccgttgggcaggggtcctgggcccacccgggcaggacgcgtggaccgagtgaccgtggtttctgtgtggtgtcacctgccagacccgccgaagaagccacctctttggagggtgcgctctctggcacgcgccactcccacccatccgtgggccgccagcaccacgcgggccccccatccacatcgcggccaccacgtccctgggacacgccttgtcccccggtgtacgccgagaccaagcacttcctctactcctcaggcgacaaggagcagctgcggccctccttcctactcagctctctgaggcccagcctgactggcgctcggaggctcgtggagaccatctttctgggttccaggccctggatgccagggactccccgcaggttgccccgcctgccccagcgctactggcaaatgcggcccctgtttctggagctgcttgggaaccacgcgcagtgcccctacggggtgctcctcaagacgcactgcccgctgcgagctgcggtcaccccagcagccggtgtctgtgcccgggagaagccccagggctctgtggcggcccccgaggaggaggacacagacccccgtcgcctggtgcagctgctccgccagcacagcagcccctggcaggtgtacggcttcgtgcgggcctgcctgcgccggctggtgcccccaggcctctggggctccaggcacaacgaacgccgcttcctcaggaacaccaagaagttcatctccctggggaagcatgccaagctctcgctgcaggagctgacgtggaagatgagcgtgcgggactgcgcttggctgcgcaggagcccaggggttggctgtgttccggccgcagagcaccgtctgcgtgaggagatcctggccaagttcctgcactggctgatgagtgtgtacgtcgtcgagctgctcaggtctttcttttatgtcacggagaccacgtttcaaaagaacaggctctttttctaccggaagagtgtctggagcaagttgcaaagcattggaatcagacagcacttgaagagggtgcagctgcgggagctgtcggaagcagaggtcaggcagcatcgggaagccaggcccgccctgctgacgtccagactccgcttcatccccaagcctgacgggctgcggccgattgtgaacatggactacgtcgtgggagccagaacgttccgcagagaaaagagggccgagcgtctcacctcgagggtgaaggcactgttcagcgtgctcaactacgagcgggcgcggcgccccggcctcctgggcgcctctgtgctgggcctggacgatatccacagggcctggcgcaccttcgtgctgcgtgtgcgggcccaggacccgccgcctgagctgtactttgtcaaggtggatgtgacgggcgcgtacgacaccatcccccaggacaggctcacggaggtcatcgccagcatcatcaaaccccagaacacgtactgcgtgcgtcggtatgccgtggtccagaaggccgcccatgggcacgtccgcaaggccttcaagagccacgtctctaccttgacagacctccagccgtacatgcgacagttcgtggctcacctgcaggagaccagcccgctgagggatgccgtcgtcatcgagcagagctcctccctgaatgaggccagcagtggcctcttcgacgtcttcctacgcttcatgtgccaccacgccgtgcgcatcaggggcaagtcctacgtccagtgccaggggatcccgcagggctccatcctctccacgctgctctgcagcctgtgctacggcgacatggagaacaagctgtttgcggggattcggcgggacgggctgctcctgcgtttggtggatgatttcttgttggtgacacctcacctcacccacgcgaaaaccttcctcagctatgcccggacctccatcagagccagtctcaccttcaaccgcggcttcaaggctgggaggaacatgcgtcgcaaactctttggggtcttgcggctgaagtgtcacagcctgtttctggatttgcaggtgaacagcctccagacggtgtgcaccaacatctacaagatcctcctgctgcaggcgtacaggtttcacgcatgtgtgctgcagctcccatttcatcagcaagtttggaagaaccccacatttttcctgcgcgtcatctctgacacggcctccctctgctactccatcctgaaagccaagaacgcagggatgtcgctgggggccaagggcgccgccggccctctgccctccgaggccgtgcagtggctgtgccaccaagcattcctgctcaagctgactcgacaccgtgtcacctacgtgccactcctggggtcactcaggacagcccagacgcagctgagtcggaagctcccggggacgacgctgactgccctggaggccgcagccaacccggcactgccctcagacttcaagaccatcctggactga

SEQ ID NO: 11 - protein, 317 aa, Homo sapiens
MFQAAERPQEWAMEGPRDGLKKERLLDDRHDSGLDSMKDEEYEQMVKELQEIRLEPQEVPRGSEPWKQQLTEDGDSFLHLAIIHEEKALTMEVIRQVKGDLAFLNFQNNLQQTPLHLAVITNQPEIAEALLGAGCDPELRDFRGNTPLHLACEQGCLASVGVLTQSCTTPHLHSILKATNYNGHTCLHLASIHGYLGIVELLVSLGADVNAQEPCNGRTALHLAVDLQNPDLVSLLLKCGADVNRVTYQGYSPYQLTWGRPSTRIQQQLGQLTLENLQMLPESEDEESYDTESEFTEFTEDELPYDDCVFGGQRLTL

SEQ ID NO: 12 - DNA, 954 bp, Homo sapiens
atgttccaggcggccgagcgcccccaggagtgggccatggagggcccccgcgacgggctgaagaaggagcggctactggacgaccgccacgacagcggcctggactccatgaaagacgaggagtacgagcagatggtcaaggagctgcaggagatccgcctcgagccgcaggaggtgccgcgcggctcggagccctggaagcagcagctcaccgaggacggggactcgttcctgcacttggccatcatccatgaagaaaaggcactgaccatggaagtgatccgccaggtgaagggagacctggctttcctcaacttccagaacaacctgcagcagactccactccacttggctgtgatcaccaaccagccagaaattgctgaggcacttctgggagctggctgtgatcctgagctccgagactttcgaggaaatacccccctacaccttgcctgtgagcagggctgcctggccagcgtgggagtcctgactcagtcctgcaccaccccgcacctccactccatcctgaaggctaccaactacaatggccacacgtgtctacacttagcctctatccatggctacctgggcatcgtggagcttttggtgtccttgggtgctgatgtcaatgctcaggagccctgtaatggccggactgcccttcacctcgcagtggacctgcaaaatcctgacctggtgtcactcctgttgaagtgtggggctgatgtcaacagagttacctaccagggctattctccctaccagctcacctggggccgcccaagcacccggatacagcagcagctgggccagctgacactagaaaaccttcagatgctgccagagagtgaggatgaggagagctatgacacagagtcagagttcacggagttcacagaggacgagctgccctatgatgactgtgtgtttggaggccagcgtctgacgttatga

SEQ ID NO: 13 - protein, 719 aa, artificial sequence
  Fusion protein
MFQAAERPQEWAMEGPRDGLKKERLLDDRHDSGLDSMKDEEYEQMVKELQEIRLEPQEVPRGSEPWKQQLTEDGDSFLHLAIIHEEKALTMEVIRQVKGDLAFLNFQNNLQQTPLHLAVITNQPEIAEALLGAGCDPELRDFRGNTPLHLACEQGCLASVGVLTQSCTTPHLHSILKATNYNGHTCLHLASIHGYLGIVELLVSLGADVNAQEPCNGRTALHLAVDLQNPDLVSLLLKCGADVNRVTYQGYSPYQLTWGRPSTRIQQQLGQLTLENLQMLPESEDEESYDTESEFTEFTEDELPYDDCVFGGQRLTLGSRQHHAGPPSTSRPPRPWDTPCPPVYAETKHFLYSSGDKEQLRPSFLLSSLRPSLTGARRLVETIFLGSRPWMPGTPRRLPRLPQRYWQMRPLFLELLGNHAQCPYGVLLKTHCPLRAAVTPAAGVCAREKPQGSVAAPEEEDTDPRRLVQLLRQHSSPWQVYGFVRACLRRLVPPGLWGSRHNERRFLRNTKKFISLGKHAKLSLQELTWKMSVRDCAWLRRSPGVGCVPAAEHRLREEILAKFLHWLMSVYVVELLRSFFYVTETTFQKNRLFFYRKSVWSKLQSIGIRQHLKRVQLRELSEAEVRQHREARPALLTSRLRFIPKPDGLRPIVNMDYVVGARTFRREKRAERLTSRVKALFSVLNYERARRPGLLGASVLGLDDIHRAWRTFVLRVRAQ

SEQ ID NO: 14 - DNA, 2160 bp, artificial sequence
  fusion construct
atgttccaggcggccgagcgcccccaggagtgggccatggagggcccccgcgacgggctgaagaaggagcggctactggacgaccgccacgacagcggcctggactccatgaaagacgaggagtacgagcagatggtcaaggagctgcaggagatccgcctcgagccgcaggaggtgccgcgcggctcggagccctggaagcagcagctcaccgaggacggggactcgttcctgcacttggccatcatccatgaagaaaaggcactgaccatggaagtgatccgccaggtgaagggagacctggccttcctcaacttccagaacaacctgcagcagactccactccacttggctgtgatcaccaaccagccagaaattgctgaggcacttctgggagctggctgtgatcctgagctccgagactttcgaggaaatacccccctacaccttgcctgtgagcagggctgcctggccagcgtgggagtcctgactcagtcctgcaccaccccgcacctccactccatcctgaaggctaccaactacaatggccacacgtgtctacacttagcctctatccatggctacctgggcatcgtggagcttttggtgtccttgggtgctgatgtcaatgctcaggagccctgtaatggccggactgcccttcacctcgcagtggacctgcaaaatcctgacctggtgtcactcctgttgaagtgtggggctgatgtcaacagagttacctaccagggctattctccctaccagctcacctggggccgcccaagcacccggatacagcagcagctgggccagctgacactagaaaaccttcagatgctgccagagagtgaggatgaggagagctatgacacagagtcagagttcacggagttcacagaggacgagctgccctatgatgactgtgtgtttggaggccagcgtctgacgttaggatcccgccagcaccacgcgggccccccatccacatcgcggccaccacgtccctgggacacgccttgtcccccggtgtacgccgagaccaagcacttcctctactcctcaggcgacaaggagcagctgcggccctccttcctactcagctctctgaggcccagcctgactggcgctcggaggctcgtggagaccatctttctgggttccaggccctggatgccagggactccccgcaggttgccccgcctgccccagcgctactggcaaatgcggcccctgtttctggagctgcttgggaaccacgcgcagtgcccctacggggtgctcctcaagacgcactgcccgctgcgagctgcggtcaccccagcagccggtgtctgtgcccgggagaagccccagggctctgtggcggcccccgaggaggaggacacagacccccgtcgcctggtgcagctgctccgccagcacagcagcccctggcaggtgtacggcttcgtgcgggcctgcctgcgccggctggtgcccccaggcctctggggctccaggcacaacgaacgccgcttcctcaggaacaccaagaagttcatctccctggggaagcatgccaagctctcgctgcaggagctgacgtggaagatgagcgtgcgggactgcgcttggctgcgcaggagcccaggggttggctgtgttccggccgcagagcaccgtctgcgtgaggagatcctggccaagttcctgcactggctgatgagtgtgtacgtcgtcgagctgctcaggtctttcttttatgtcacggagaccacgtttcaaaagaacaggctctttttctaccggaagagtgtctggagcaagttgcaaagcattggaatcagacagcacttgaagagggtgcagctgcgggagctgtcggaagcagaggtcaggcagcatcgggaagccaggcccgccctgctgacgtccagactccgcttcatccccaagcctgacgggctgcggccgattgtgaacatggactacgtcgtgggagccagaacgttccgcagagaaaagagggccgagcgtctcacctcgagggtgaaggcactgttcagcgtgctcaactacgagcgggcgcggcgccccggcctcctgggcgcctctgtgctgggcctggacgatatccacagggcctggcgcaccttcgtgctgcgtgtgcgggcccagtga

SEQ ID NO: 15 - protein, 365 aa, Homo sapiens [sequence omitted]

SEQ ID NO: 16 - protein, 498 aa, artificial sequence
  fusion protein
MAHFPGFGQSLLYGYPVYVFGDCVQADWCPVSGGLCSTRLHRHALLATCPEHQLTWDPIDGRVVSSPLQYLIPRLPSFPTQRTSRTLKVLTPPTTPVSPKVPPAFFQSMRKHTPYRNGCLEPTLGDQLPSLAFPEPGLRPQNIYTTWGKTVVCLYLYQLSPPMTWPLIPHVIFCHPRQLGAFLTKVPLKRLEELLYKMFLHTGTVIVLPVDDLPTTMFQPVRAPCIQTAWCTGLLPYHSILTTPGLIWTFNDGSPMISGPCPKAGQPSLVVQSSLLIFEKFQTKAFHPSYLLSHQLIQYSSFHNLHLLFDEYTNIPVSILFNKEEADDNGDGSVSKGEELFTGVVPILVELDGDVNGHKFSVSGEGEGDATYGKLTLKFICTTGKLPVPWPTLVTTLTYGVQCFSRYPDHMKQHDFFKSAMPEGYVQERTIFFKDDGNYKTRAEVKFEGDTLVNRIELKGIDFKEDGNILGHKLEYNYNSHNVYIMADKQKNGIKVNF

SEQ ID NO: 17 - DNA, 1497 bp, artificial sequence
  fusion construct
atggcccatttcccaggatttggacaaagcctcctatatggataccccgtctacgtgtttggcgattgtgtacaggccgattggtgtcccgtctcaggtggtctatgttccacccgcctacatcgacatgccctcctggccacctgtccagagcaccaactcacctgggaccccatcgatggacgcgttgtcagctctcctctccaataccttatccctcgcctcccctccttccccacccagagaacctcaaggaccctcaaggtccttacccctcccaccactcctgtctcccccaaggttccacctgccttctttcaatcaatgcgaaagcacaccccctaccgaaatggatgcctggaaccaaccctcggggatcagctcccctccctcgccttccccgaacctggcctccgtccccaaaacatctacaccacctggggaaaaaccgtagtatgcctatacctataccagctttccccacccatgacatggccacttataccccatgtcatattctgccaccccagacaattaggagccttcctcaccaaggtgcctctaaaacgattagaagaacttctatacaaaatgttcctacacacagggacagtcatagtcctcccagtggacgacctacccaccacaatgttccaacccgtgagggctccctgtatccagactgcctggtgtacaggacttctcccctatcactccatcttaacaaccccaggtctaatatggaccttcaatgacggctcaccaatgatttccggcccttgccccaaagcagggcagccatctttagtagttcagtcctccctattaatcttcgaaaaattccaaaccaaagccttccatccctcctatctactctctcatcagcttatacaatactcctccttccataaccttcaccttctattcgatgaatacaccaacatccctgtctctattttatttaataaagaagaggcggatgacaatggcgacggatccgtgagcaagggcgaggagctgttcaccggggtggtgcccatcctggtcgagctggacggcgacgtaaacggccacaagttcagcgtgtccggcgagggcgagggcgatgccacctacggcaagctgaccctgaagttcatctgcaccaccggcaagctgcccgtgccctggcccaccctcgtgaccaccctgacctacggcgtgcagtgcttcagccgctaccccgaccacatgaagcagcacgacttcttcaagtccgccatgcccgaaggctacgtccaggagcgcaccatcttcttcaaggacgacggcaactacaagacccgcgccgaggtgaagttcgagggcgacaccctggtgaaccgcatcgagctgaagggcatcgacttcaaggaggacggcaacatcctggggcacaagctggagtacaactacaacagccacaacgtctatatcatggccgacaagcagaagaacggcatcaaggtgaacttctaa

SEQ ID NO: 18 - DNA, 24 bp, artificial sequence
  probe
gatccttctgggaattcctagatc

SEQ ID NO: 19 - DNA, 25 bp, artificial sequence
  probe
gatccggcaggggaatctccctctc

SEQ ID NO: 20 - DNA, 21 bp, artificial sequence
  probe
cgcttgatgactcagccggaa

SEQ ID NO: 21 - DNA, 20 bp, artificial sequence
  primer
gcaccgtcaaggctgagaac

SEQ ID NO: 22 - DNA, 19 bp, artificial sequence
  primer
tggtgaagacgccagtgga

SEQ ID NO: 23 - DNA, 20 bp, artificial sequence
  primer
cagtgctgctgaaggagatg

SEQ ID NO: 24 - DNA, 20 bp, artificial sequence
  primer
aacaagtttggatgggcaac

SEQ ID NO: 25 - DNA, 20 bp, artificial sequence
  primer
tggcaatgaggatgacttgt

SEQ ID NO: 26 - DNA, 19 bp, artificial sequence
  primer
tggtggtcggagattcgta

SEQ ID NO: 27 - DNA, 22 bp, artificial sequence
  primer
ctcaccaggatgctcacattta

SEQ ID NO: 28 - DNA, 22 bp, artificial sequence
  primer
cctccagaggtttgagttcttc

SEQ ID NO: 29 - DNA, 19 bp, artificial sequence
  primer
ggagacttgcctggtgaaa

SEQ ID NO: 30 - DNA, 21 bp, artificial sequence
  primer
ctggcttgttcctcactactc

SEQ ID NO: 31 - DNA, 18 bp, artificial sequence
  primer
ctggccgtggctctcttg

SEQ ID NO: 32 - DNA, 20 bp, artificial sequence
  primer
ccttggcaaaactgcacctt

SEQ ID NO: 33 - DNA, 20 bp, artificial sequence
  primer
tttccctgacctccctctaa

SEQ ID NO: 34 - DNA, 22 bp, artificial sequence
  primer
cgagacactggaaggtgaatta

SEQ ID NO: 35 - DNA, 22 bp, artificial sequence
  primer
ccttgtggctaccctggtcctc

SEQ ID NO: 36 - DNA, 22 bp, artificial sequence
  primer
ctcagcaggttttgggagtggt

SEQ ID NO: 37 - DNA, 20 bp, artificial sequence
  primer
accagagcagtgaggtctta

SEQ ID NO: 38 - DNA, 22 bp, artificial sequence
  primer
ctcctttgtgacaggtgtactg

SEQ ID NO: 39 - DNA, 22 bp, artificial sequence
  primer
gagtccggagatgcaagtattc

SEQ ID NO: 40 - DNA, 22 bp, artificial sequence
  primer
cctccagttcctcacattcttt

SEQ ID NO: 41 - DNA, 20 bp, artificial sequence
  primer
acccacagcctggataacag

SEQ ID NO: 42 - DNA, 20 bp, artificial sequence
  primer
actggttgccatcaaactcc

SEQ ID NO: 43 - DNA, 22 bp, artificial sequence
  primer
tcaatctcttcagcacaaagga

SEQ ID NO: 44 - DNA, 20 bp, artificial sequence
  primer
atcacacaggcttccaggtc

SEQ ID NO: 45 - DNA, 20 bp, artificial sequence
  primer
tctcctgttgtgcttctcca

SEQ ID NO: 46 - DNA, 22 bp, artificial sequence
  primer
gtcaaagttcatcctgtccttg

SEQ ID NO: 47 - DNA, 20 bp, artificial sequence
  primer
gccgaattccggatctacaa

SEQ ID NO: 48 - DNA, 21 bp, artificial sequence
  primer
ctcctggagcacctgataaac

SEQ ID NO: 49 - DNA, 22 bp, artificial sequence
  primer
cccatgggttgtgtgtttattt

SEQ ID NO: 50 - DNA, 21 bp, artificial sequence
  primer
aaaccggcagtaactggatag

SEQ ID NO: 51 - DNA, 22 bp, artificial sequence
  primer
gatccctgacatctggaatctg

SEQ ID NO: 52 - DNA, 22 bp, artificial sequence
  primer
gaaacatctggagagaggaagg

SEQ ID NO: 53 - DNA, 20 bp, artificial sequence
  primer
cagaggaggaacgagctaaa

SEQ ID NO: 54 - DNA, 20 bp, artificial sequence
  primer
ttggacggacaggatgtatg